European Patent Application EP 4 592 385 A1, published July 30, 2025. Title: IMINE REDUCTASE MUTANT, APPLICATION THEREOF AND APPLICATION METHOD THEREFOR. Applicant: Zhejiang Ano Bio-pharmaceutical Co.,Ltd. The sequence listing filed with the application follows.

SEQUENCE LISTING (12 sequences)

SEQ ID NO: 1 - protein, 287 aa, Artificial Sequence
MKTPVTVLGLGAMGRALVTALLDAGRPVTVWNRTPGKADELAGAVEAASVHDAVTAGGIVVVCLYDHASVHETLDPVAAGLRGRAVVNLTTTTPAEARELAEWADGHGIEYLDGAIMATPPMIGAPGAQILYSGSRAVFDGHREALDLWATSVYDGADAGMASLFDLAILSGMYPLFAGFLHGAAMVRAEGVPAAEFAERAAPFLAAMTGSFAGIARTVDGGGYDVPGQSLDWTAGALEAIGRASREQGVDPVPVDMVGALVRRQIDEGYGSEDMSRLIESMTGDAV

SEQ ID NO: 2 - protein, 287 aa, Artificial Sequence
MKTPVTVLGLGAMGRALVTALLDAGRPVTVWNRTPGKADELAVAVEAASVHDAVTAGGIVVVCLYDHASVHETLDPVAAGLRGRAVVNLTTTTPAEARELAEWADGHGIEYLDGAIMATPPMIGAPGAQILYSGSRAVFDGHREALDLWATSVYDGADAGMASLFDLAILSGMYPLFAGFLHGAAMVRAEGVPAAEFAERAAPFLAAMTGSFAGIARTVDGGGYDVPGQSLDWTAGALEAIGRASREQGVDPVPVDMVGALVRRQIDEGYGSEDMSRLIESMTGDAV

SEQ ID NO: 3 - protein, 287 aa, Artificial Sequence
MKTPVTVLGLGAMGRALVTALLDAGRPVTVWNRTPGKADELAGAVEAASVHDAVTAGGIVVVCLYDHASVHETLDPVAAGLRGRAVVNVTTTTPAEARELAEWADGHGIEYLDGAIMATPPMIGAPGAQILYSGSRAVFDGHREALDLWATSVYDGADAGMASLFDLAILSGMYPLFAGFLHGAAMVRAEGVPAAEFAERAAPFLAAMTGSFAGIARTVDGGGYDVPGQSLDWTAGALEAIGRASREQGVDPVPVDMVGALVRRQIDEGYGSEDMSRLIESMTGDAV

SEQ ID NO: 4 - protein, 287 aa, Artificial Sequence
MKTPVTVLGLGAMGRALVTALLDAGRPVTVWNRTPGKADELAVAVEAASVHDAVTAGGIVVVCLYDHASVHETLDPVAAGLRGRAVVNVTTTTPAEARELAEWADGHGIEYLDGAIMATPPMIGAPGAQILYSGSRAVFDGHREALDLWATSVYDGADAGMASLFDLAILSGMYPLFAGFLHGAAMVRAEGVPAAEFAERAAPFLAAMTGSFAGIARTVDGGGYDVPGQSLDWTAGALEAIGRASREQGVDPVPVDMVGALVRRQIDEGYGSEDMSRLIESMTGDAV

SEQ ID NO: 5 - DNA, 864 bp, Artificial Sequence
  source 1..864: mol_type = genomic DNA
atgaagacccccgtgaccgtgctcgggctgggtgcgatgggacgtgcgctggtcaccgcgctgctcgacgcggggcggccggtcaccgtgtggaaccggacgcccgggaaggcggacgaactggcgggcgcggtcgaggccgcgagcgtccacgacgcggtgaccgcgggcgggatcgtggtcgtgtgcctctacgaccacgcctcggtgcacgagacactcgacccggtggccgccgggctgcgcggacgggcggtggtgaacctcacgaccacgacgcccgccgaggcacgggagctcgcggagtgggcggacggccacggaatcgagtacctcgacggagcgatcatggcgacgccgccgatgatcggtgctccgggcgcgcagatcctctacagcgggtcgcgtgcggtgttcgatgggcatcgcgaggcgctcgacctgtgggcgacgtccgtctacgacggtgcggacgccggaatggcgtcgctgttcgacctcgcgatcctttcgggcatgtatccgctgttcgccggattcctgcacggcgccgcgatggtccgcgccgagggcgtcccggcggccgagttcgcggagcgcgccgcgcctttcctcgccgcgatgaccgggtcgttcgccggcatcgcgcgaaccgtggacggcggcggctacgacgtgccggggcagagcctcgactggacggccggcgcgctggaggccatcggccgtgcgagccgcgagcagggcgtcgatccggttccggtcgacatggtgggggcgctcgtccggcggcagatcgacgaagggtacgggagcgaagatatgtcccggctcatcgagagcatgaccggtgacgcggtgtga

SEQ ID NO: 6 - DNA, 864 bp, Artificial Sequence
  source 1..864: mol_type = genomic DNA
atgaagacccccgtgaccgtgctcgggctgggtgcgatgggacgtgcgctggtcaccgcgctgctcgacgcggggcggtcggtcaccgtgtggaaccggacgcccgggaaggcggacgaactggcgggcgcggtcgaggccgcgagcgtccacgacgcggtgaccgcgggcgggatcgtggtcgtgtgcctctacgaccacgcctcggtgcacgagacactcgacccggtggccgccgggctgcgcggacgggcggtggtgaacctcacgaccacgacgcccgccgaggcacgggagctcgcggagtgggcggacggccacggaatcgagtacctcgacggagcgatcatggcgacgccgccgatgatcggtgctccgggcgcgcagatcctctacagcgggtcgcgtgcggtgttcgatgggcatcgcgaggcgctcgacctgtgggcgacgtccgtctacgacggtgcggacgccggaatggcgtcgctgttcgacctcgcgatcctttcgggcatgtatccgctgttcgccggattcctgcacggcgccgcgatggtccgcgccgagggcgtcccggcggccgagttcgcggagcgcgccgcgcctttcctcgccgcgatgaccgggtcgttcgccggcatcgcgcgaaccgtggacggcggcggctacgacgtgccggggcagagcctcgactggacggccggcgcgctggaggccatcggccgtgcgagccgcgagcagggcgtcgatccggttccggtcgacatggtgggggcgctcgtccggcggcagatcgacgaagggtacgggagcgaagatatgtcccggctcatcgagagcatgaccggtgacgcggtgtga

SEQ ID NO: 7 - DNA, 864 bp, Artificial Sequence
  source 1..864: mol_type = genomic DNA
atgaagacccccgtgaccgtgctcgggctgggtgcgatgggacgtgcgctggtcaccgcgctgctcgacgcggggcggccggtcaccgtgtggaaccggacgcccgggaaggcggacgaactggcgggcgcggtcgaggccgcgagcgtccacgacgcggtgaccgcgggcgggatcgtggtcgtgtgcctctacgtccacgcctcggtgcacgagacactcgacccggtggccgccgggctgcgcggacgggcggtggtgaacctcacgaccacgacgcccgccgaggcacgggagctcgcggagtgggcggacggccacggaatcgagtacctcgacggagcgatcatggcgacgccgccgatgatcggtgctccgggcgcgcagatcctctacagcgggtcgcgtgcggtgttcgatgggcatcgcgaggcgctcgacctgtgggcgacgtccgtctacgacggtgcggacgccggaatggcgtcgctgttcgacctcgcgatcctttcgggcatgtatccgctgttcgccggattcctgcacggcgccgcgatggtccgcgccgagggcgtcccggcggccgagttcgcggagcgcgccgcgcctttcctcgccgcgatgaccgggtcgttcgccggcatcgcgcgaaccgtggacggcggcggctacgacgtgccggggcagagcctcgactggacggccggcgcgctggaggccatcggccgtgcgagccgcgagcagggcgtcgatccggttccggtcgacatggtgggggcgctcgtccggcggcagatcgacgaagggtacgggagcgaagatatgtcccggctcatcgagagcatgaccggtgacgcggtgtga

SEQ ID NO: 8 - DNA, 864 bp, Artificial Sequence
  source 1..864: mol_type = genomic DNA
atgaagacccccgtgaccgtgctcgggctgggtgcgatgggacgtgcgctggtcaccgcgctgctcgacgcggggcggtcggtcaccgtgtggaaccggacgcccgggaaggcggacgaactggcgggcgcggtcgaggccgcgagcgtccacgacgcggtgaccgcgggcgggatcgtggtcgtgtgcctctacgtccacgcctcggtgcacgagacactcgacccggtggccgccgggctgcgcggacgggcggtggtgaacctcacgaccacgacgcccgccgaggcacgggagctcgcggagtgggcggacggccacggaatcgagtacctcgacggagcgatcatggcgacgccgccgatgatcggtgctccgggcgcgcagatcctctacagcgggtcgcgtgcggtgttcgatgggcatcgcgaggcgctcgacctgtgggcgacgtccgtctacgacggtgcggacgccggaatggcgtcgctgttcgacctcgcgatcctttcgggcatgtatccgctgttcgccggattcctgcacggcgccgcgatggtccgcgccgagggcgtcccggcggccgagttcgcggagcgcgccgcgcctttcctcgccgcgatgaccgggtcgttcgccggcatcgcgcgaaccgtggacggcggcggctacgacgtgccggggcagagcctcgactggacggccggcgcgctggaggccatcggccgtgcgagccgcgagcagggcgtcgatccggttccggtcgacatggtgggggcgctcgtccggcggcagatcgacgaagggtacgggagcgaagatatgtcccggctcatcgagagcatgaccggtgacgcggtgtga

SEQ ID NO: 9 - protein, 261 aa, Artificial Sequence
MYPDLKGKVVAITGAASGLGKAMAIRFGKEQAKVVINYYSNKQDPNEVKEEVIKAGGEAVVVQGDVTKEEDVKNIVQTAIKEFGTLDIMINNAGLENPVPSHEMPLKDWDKVIGTNLTGAFLGSREAIKYFVENDIKGNVINMSSVHEVIPWPLFVHYAASKGGIKLMTETLALEYAPKGIRVNNIGPGAINTPINAEKFADPKQKADVESMIPMGYIGEPEEIAAVAAWLASKEASYVTGITLFADGGMTQYPSFQAGRG

SEQ ID NO: 10 - DNA, 786 bp, Artificial Sequence
  source 1..786: mol_type = genomic DNA
atgtatccggatctgaaaggcaaggtggtggccattaccggtgccgcgagtggtctgggtaaagcgatggccatccgcttcggcaaggagcaagccaaggtggtgatcaactactacagcaacaagcaagatccgaacgaagtgaaagaagaagtgatcaaagccggtggtgaagcggttgtggttcaaggcgacgtgaccaaagaagaagacgtgaagaacatcgtgcagacggcgatcaaggagttcggcacgctggacatcatgatcaacaacgccggtctggaaaacccagtgccaagccacgagatgccgctgaaggattgggataaggtgatcggcaccaatctgacgggcgcgtttctgggtagccgtgaggcgatcaagtacttcgtggagaacgacatcaagggcaacgtgattaacatgagcagcgtgcacgaggtgatcccgtggccgctgttcgtgcattacgccgcgagcaagggcggcattaaactcatgaccgaaacgctggcgctggaatatgccccgaaaggcatccgcgtgaataacatcggcccgggcgccatcaacaccccgatcaatgcggagaagttcgccgatccgaaacagaaggccgacgtggaaagcatgatcccaatgggctacatcggcgaaccagaggaaattgcggccgttgccgcgtggctggccagcaaagaagcgagctacgttaccggtatcacgctgtttgccgatggcggcatgacgcagtatccgagtttccaagccggtcgcggctaa

SEQ ID NO: 11 - DNA, 30 bp, Artificial sequence
  source 1..30: mol_type = genomic DNA
acatacatgtaatgaagccagacggtgtga

SEQ ID NO: 12 - DNA, 30 bp, Artificial sequence
  source 1..30: mol_type = genomic DNA
aggtcctagcgttaagccgcacgcagttcc